European Patent Application EP 4 317 425 A1, published February 7, 2024. Title: PPO polypeptides tolerant to PPO-inhibiting herbicides and use thereof. Applicant: QINGDAO KINGAGROOT CHEMICAL COMPOUND CO., LTD. The sequence listing filed with the application follows.

SEQUENCE LISTING (49 sequences)

SEQ ID NO: 1 - protein, 536 aa, Artificial sequence
  Amino-acid sequence of PPO1 from wild-type rice (OsPPO1 WT)
MAAAAAAMATATSATAAPPLRIRDAARRTRRRGHVRCAVASGAAEAPAAPGARVSADCVVVGGGISGLCTAQALATKHGVGDVLVTEARARPGGNITTAERAGEGYLWEEGPNSFQPSDPVLTMAVDSGLKDDLVFGDPNAPRFVLWEGKLRPVPSKPGDLPFFDLMSIPGKLRAGLGALGVRAPPPGREESVEDFVRRNLGAEVFERLIEPFCSGVYAGDPSKLSMKAAFGKVWRLEDTGGSIIGGTIKTIQERGKNPKPPRDPRLPTPKGQTVASFRKGLTMLPDAITSRLGSKVKLSWKLTSITKSDNKGYALVYETPEGVVSVQAKTVVMTIPSYVASDILRPLSSDAADALSIFYYPPVAAVTVSYPKEAIRKECLIDGELQGFGQLHPRSQGVETLGTIYSSSLFPNRAPAGRVLLLNYIGGSTNTGIVSKTESELVEAVDRDLRKMLINPKAVDPLVLGVRVWPQAIPQFLIGHLDHLEAAKSALGKGGYDGLFLGGNYVAGVALGRCVEGAYESASQISDYLTKYAYK

SEQ ID NO: 2 - protein, 537 aa, Artificial sequence
  Amino-acid sequence of PPO1 from wild-type corn (ZmPPO1 WT)
MVAATATATAMATAASPLLNGTRIPARLRHRGLSVRCAAVAGGAAEAPASTGARLSADCVVVGGGISGLCTAQALATRHGVGDVLVTEARARPGGNITTVERPEEGYLWEEGPNSFQPSDPVLTMAVDSGLKDDLVFGDPNAPRFVLWEGKLRPVPSKPADLPFFDLMSIPGKLRAGLGALGIRPPPPGREESVEEFVRRNLGAEVFERLIEPFCSGVYAGDPSKLSMKAAFGKVWRLEETGGSIIGGTIKTIQERSKNPKPPRDARLPKPKGQTVASFRKGLAMLPNAITSSLGSKVKLLWKLTSITKSDDKGYVLEYETPEGVVSVQAKSVIMTIPSYVASNILRPLSSDAADALSRFYYPPVAAVTVSYPKEAIRKECLIDGELQGFGQLHPRSQGVETLGTIYSSSLFPNRAPDGRVLLLNYIGGATNTGIVSKTESELVEAVDRDLRKMLINSTAVDPLVLGVRVWPQAIPQFLVGHLDLLEAAKAALDRGGYDGLFLGGNYVAGVALGRCVEGAYESASQISDFLTKYAYK

SEQ ID NO: 3 - protein, 537 aa, Artificial sequence
  Amino-acid sequence of PPO1 wild-type from oilseed rape (BnPPO1-C5)
MDLSLLRPQPFLSPFSNPFPRSRPYKPPNLRCSVSGGSVVGGSSTIEGGRGGKTVAADCVIVGGGISGLCIAQALVTKHPDAAKSVMVTEAKDRVGGNIITREEQGFLWEEGPNSFQPSDPMLTMVVDSGLKDDLVLGDPTAPRFVLWNGKLRPVPSKLTDLPFFDLMSIGGKIRAGFGAIGIRPSPPGREESVEEFVRRNLGDEVFERLIEPFCSGVYAGDPAKLSMKAAFGKVWKLEENGGSIIGGAFKAIQARNKAPKTTRDPRLPKPKGQTVGSFRKGLTMLPDAISARLGDKVKVSWKLSSISKLPSGGYSLTYETPEGIVTVQSKSVVMTVPSHVASSLLRPLSDSAAEALSKLYYPPVAAVSISYPKEAIRSECLIDGELKGFGQLHPRTQKVETLGTIYSSSLFPNRAPPGRVLLLNYIGGATNTGILSKSEGELVEAVDRDLRKMLIKPSSTDPLVLGVKVWPQAIPQFLIGHIDLVDAAKASLSSSGHEGLFLGGNYVAGVALGRCVEGAYETATQVNDFMSRYAYK

SEQ ID NO: 4 - protein, 536 aa, Artificial sequence
  Amino-acid sequence of PPO1 from wild-type oilseed rape (BnPPO1-A10)
MDLSLLRPQPFLSPFSNPFPRSRPYKPLNLRCSVSGGSVVGSSTIEGGGGGKTVTADCVIVGGGISGLCIAQALVTKHPDAAKNVMVTEAKDRVGGNIITREEQGFLWEEGPNSFQPSDPMLTMVVDSGLKDDLVLGDPTAPRFVLWNGKLRPVPSKLTDLPFFDLMSIGGKIRAGFGAIGIRPSPPGREESVEEFVRRNLGDEVFERLIEPFCSGVYAGDPAKLSMKAAFGKVWKLEENGGSIIGGAFKAIQAKNKAPKTTRDPRLPKPKGQTVGSFRKGLTMLPEAISARLGDKVKVSWKLSSITKLASGEYSLTYETPEGIVTVQSKSVVMTVPSHVASSLLRPLSDSAAEALSKLYYPPVAAVSISYAKEAIRSECLIDGELKGFGQLHPRTQKVETLGTIYSSSLFPNRAPPGRVLLLNYIGGATNTGILSKSEGELVEAVDRDLRKMLIKPSSTDPLVLGVKLWPQAIPQFLIGHIDLVDAAKASLSSSGHEGLFLGGNYVAGVALGRCVEGAYETATQVNDFMSRYAYK

SEQ ID NO: 5 - protein, 558 aa, Artificial sequence
  Amino-acid sequence of PPO1 from wild-type peanut (AhPPO1-A)
MPAMLTLPNDTVFLQNTMHSPTSSFSPHSPLIIPFPSPCRHPSTTKFPLIRCSLAGESSTASPAKPAALPRSAVGASVDCVVVGGGISGLCIAQALSTKHAKAAANVVVTEARDRVGGNITTIERDGYLWEEGPNSFQPSDPMLTMVVDSGLKDELVLGDPNAPRFVLWNGELRPVPGKPTDLPFFDLMSFGGKLRAGFGALGIRPPPPGHEESVEEFVRRNLGDEVFERLIEPFCSGVYAGDPSKLSMKAAFGKVWRLEQNGGSIIGGTFKAIQERKSTSKPPRDPRLPTPKGQTVGSFRKGLTMLPEAISAKLGNKVKLSWKLLGISKLDSGEYSLTYDTPEGVVSLQTKSVVMTIPSHVASTLLRSISDAAADALSKFYYPPVAAVSVSYPKEAIRSECLIDGELKGFGQLHPRTQGVETLGTIYSSSLFPNRAPDGRVLLLNYIGGATNPGILSKTDSELVEAVDRDLRKMLINPNAGDPFALGVRVWPQAIPQFLVGHLDLLDIAKSSLKNTGFEGLFLGGNYVSGVALGRCVEGAYEIAAEVDDFLAQKVYK

SEQ ID NO: 6 - protein, 552 aa, Artificial sequence
  Amino-acid sequence of PPO1 from wild-type peanut (AhPPO1-B)
MSAMLTLPNDTVFLQNTMHSPTSSFSPHSPLIIPFPSPCRHPSTTKFPLIRCSLAGESSTASLPRSAVGASVDCVVVGGGISGLCIAQALSTKHAKAAANVVVTEARDRVGGNITTVERDGYLWEEGPNSFQPSDPMLTMVVDSGLKDELVLGDPNAPRFVLWNGRLRPVPGKPTDLPFFDLMSFGGKLRAGFGALGIRPPPPGHEESVEEFVRRNLGDEVFERLIEPFCSGVYAGDPSKLSMKAAFGKVWRLEQNGGSIIGGTFKAIQERKSTSKPPRDPRLPTPKGQTVGSFRKGLIMLPEAISAKLGNKVKLSWKLLGISKLDSGEYSLTYDTPEGVVSLQTKSVVMTIPSHVASTLLRSISETAADALSKFYYPPVAAVSVSYPKEAIRSECLIDGELKGFGQLHPRTQGVETLGTIYSSSLFPNRAPDGRVLLLNYIGGATNPGILSKTDSELVEAVDRDLRKMLINPNAGDPFALGVRVWPQAIPQFLVGHLDLLDIAKSSLKNTGFEGLFLGGNYVSGVALGRCVEGAYEIAAEVDDFLAQKVYK

SEQ ID NO: 7 - protein, 543 aa, Artificial sequence
  Amino-acid sequence of PPO1 from wild-type soybean (GmPPO1)
MVSVFNEILFPPNQTLLRPSLHSPTSFFTSPTRKFPRSRPNPILRCSIAEESTASPPKTRDSAPVDCVVVGGGVSGLCIAQALATKHANANVVVTEARDRVGGNITTMERDGYLWEEGPNSFQPSDPMLTMVVDSGLKDELVLGDPDAPRFVLWNRKLRPVPGKLTDLPFFDLMSIGGKIRAGFGALGIRPPPPGHEESVEEFVRRNLGDEVFERLIEPFCSGVYAGDPSKLSMKAAFGKVWKLEKNGGSIIGGTFKAIQERNGASKPPRDPRLPKPKGQTVGSFRKGLTMLPDAISARLGNKVKLSWKLSSISKLDSGEYSLTYETPEGVVSLQCKTVVLTIPSYVASTLLRPLSAAAADALSKFYYPPVAAVSISYPKEAIRSECLIDGELKGFGQLHPRSQGVETLGTIYSSSLFPNRAPPGRVLLLNYIGGATNTGILSKTDSELVETVDRDLRKILINPNAQDPFVVGVRLWPQAIPQFLVGHLDLLDVAKASIRNTGFEGLFLGGNYVSGVALGRCVEGAYEVAAEVNDFLTNRVYK

SEQ ID NO: 8 - protein, 536 aa, Artificial sequence
  Amino-acid sequence of PPO1 from wild-type sorghum(SbPPO1)
MVAAAAMATAASAAAPLLNGTRRPARLRRRGLRVRCAAVAGGAAEAPASTGARLSADCVVVGGGISGLCTAQALATRHGVGEVLVTEARARPGGNITTVERPEEGYLWEEGPNSFQPSDPVLSMAVDSGLKDDLVFGDPNAPRFVLWEGKLRPVPSKPADLPFFDLMSIPGKLRAGLGALGIRPPPPGREESVEEFVRRNLGAEVFERLIEPFCSGVYAGDPSKLSMKAAFGKVWRLEEAGGSIIGGTIKTIQERGKNPKPPRDPRLPKPKGQTVASFRKGLAMLPNAITSSLGSKVKLSWKLTSITKSDGKGYVLEYETPEGVVLVQAKSVIMTIPSYVASDILRPLSGDAADALSRFYYPPVAAVTVSYPKEAIRKECLIDGELQGFGQLHPRSQGVETLGTIYSSSLFPNRAPAGRVLLLNYIGGATNTGIVSKTESELVEAVDRDLRKMLINSTAVDPLVLGVRVWPQAIPQFLVGHLDLLEVAKSALDQGGYDGLFLGGNYVAGVALGRCIEGAYESAAQIYDFLTKYAYK

SEQ ID NO: 9 - protein, 531 aa, Artificial sequence
  Amino-acid sequence of PPO1 from wild-type wheat (TaPPO1-A)
MAGATMATATVTAASPLRGRVTGRPRRVRTRCAAASGATETPAAPGVRLSAECVIVGAGISGLCTAQALATRYGVSDLLVTEARDRPGGNITTVERPDEGYLWEEGPNSFQPSDPVLTMAVDSGLKDDLVFGDPNAPRFVLWEGKLRPVPSKPGDLPFFSLMSIPGKLRAGLGALGIRPPPPGREESVEEFVRRNLGAEVFERLIEPFCSGVYAGDPSKLSMKAAFGKVWRLEEIGGSIIGGTIKAIQDKGKNPKPPRDPRLPAPKGQTVASFRKGLAMLPNAIASRLGSKVKLSWKLTSITKADNQGYVLGYETPEGLVSVQAKSVIMTIPSYVASDILRPLSIDAADALSKFYYPPVAAVTVSYPKEAIRKECLIDGELQGFGQLHPRSQGVETLGTIYSSSLFPNRAPAGRVLLLNYIGGSTNTGIVSKTESDLVEAVDRDLRKMLINPRAADPLALGVRVWPQAIPQFLIGHLDRLAAAKSALGRGGYDGLFLGGNYVAGVALGRCIEGAYESASQVSDFLTKYAYK

SEQ ID NO: 10 - protein, 531 aa, Artificial sequence
  Amino-acid sequence of PPO1 from wild-type wheat (TaPPO1-B)
MAGATMATATVAAASPLRGRVTGRPHRVRPRCATASSATETPAAPGVRLSAECVIVGAGISGLCTAQALATRYGVSDLLVTEARDRPGGNITTVERPDEGYLWEEGPNSFQPSDPVLTMAVDSGLKDDLVFGDPNAPRFVLWEGKLRPVPSKPGDLPFFSLMSIPGKLRAGLGALGIRPPPPGREESVEEFVRRNLGAEVFERLIEPFCSGVYAGDPSKLSMKAAFGKVWRLEEIGGSIIGGTIKAIQDKGKNPKPPRDPRLPAPKGQTVASFRKGLAMLPNAIASRLGSKVKLSWKLTSITKADNQGYVLGYETPEGLVSVQAKSVIMTIPSYVASDILRPLSIDAADALSKFYYPPVAAVTVSYPKEAIRKECLIDGELQGFGQLHPRSQGVETLGTIYSSSLFPNRAPAGRVLLLNYIGGSTNTGIVSKTESDLVGAVDRDLRKMLINPRAADPLALGVRVWPQAIPQFLIGHLDRLAAAKSALGQGGYDGLFLGGNYVAGVALGRCIEGAYESASQVSDFLTKYAYK

SEQ ID NO: 11 - protein, 531 aa, Artificial sequence
  Amino-acid sequence of PPO1 from wild-type wheat (TaPPO1-D)
MAGATMATATVTAASPLRGRVTGRPRRVRPRCAAASGATETPAAPGVRLSADCVIVGAGISGLCTAQALATRYGVGDLLITEARDRPGGNITTVERPDEGYLWEEGPNSFQPSDPVLTMAVDSGLKDDLVFGDPNAPRFVLWEGKLRPVPSKPGDLPFFSLMSIPGKLRAGLGALGIRPPPPGREESVEEFVRRNLGAEVFERLIEPFCSGVYAGDPSKLSMKAAFGKVWRLEEIGGSIIGGTIKAIQDKGKNPKPPRDPRLPAPKGQTVASFRKGLAMLPNAIASRLGSKVKLSWKLTSITKADNQGYVLGYETPEGLVSVQAKSVIMTIPSYVASDILRPLSIDAADALSKFYYPPVAAVTVSYPKEAIRKECLIDGELQGFGQLHPRSQGVETLGTIYSSSLFPNRAPAGRVLLLNYIGGSTNTGIVSKTESDLVEAVDSDLRKMLINPRAADPLALGVRVWPQAIPQFLIGHLDRLAAAKSALGRGGYDGLFLGGNYVAGVALGRCIEGAYESASQVSDFLTKYAYK

SEQ ID NO: 12 - protein, 558 aa, Artificial sequence
  Amino-acid sequence of PPO1 form wild-type tomato (SlPPO1)
MTTTAVVNHPSIFTHRSPLPSPSSSSSSSPSFLFLNRTNFIPYFSTSKRSSVNCNGWRTRCSVAKNYTVPPSEVDGNQLPELDCVVVGAGISGLCIAKVISANYPNLMVTEARDRAGGNITTVERDGYLWEEGPNSFQPSDPMLTMAVDCGLKDDLVLGDPDAPRFVLWKDKLRPVPGKLTDLPFFDLMSIPGKLRAGFGAIGLRPSPPGYEESVEQFVRRNLGAEVFERLIESFCSGVYAGDPSKLSMKAAFGKVWKLEQTGGSIIGGTFKAIKERSSNPKPPRDPRLPTPKGQTVGSFRKGLRMLPDAICERLGSKVKLSWKLSSITKSDKGGYLLTYETPEGVVSLRSRSIVMTVPSYVASNILRPLSVAAADALSSFYYPPVAAVTISYPQEAIRDERLVDGELKGFGQLHPRSQGVETLGTIYSSSLFPNRAPNGRVLLLNYIGGATNTEIVSKTESQLVEAVDRDLRKMLIKPKAQDPFVTGVRVWPQAIPQFLVGHLDTLGTAKAALSDNGLDGLFLGGNYVSGVALGRCVEGAYEIASEVTGFLSQYAYK

SEQ ID NO: 13 - protein, 557 aa, Artificial sequence
  Amino-acid sequence of PPO1 from wild-type potato (StPPO1)
MTTTAVANHPSIFTHRSPLLSPSSSSSSPSFLFLNRTNFIPYFSTSKRNSVNCNGWRTRCSVAKDYTVPPSEVDGNQFPELDCVVVGAGISGLCITKVISDNYPNLMVTEARDRAGGNITTVERDGYLWEEGPNSFQPSDPMLTMAVDCGLKDDLVLGDPDAPRFVLWKDKLRPVPGKLTDLPFFDLMSIPGKLRAGFGAIGLRPSPPGYEESVEQFVRRNLGAEVFERLIEPFCSGVYAGDPSKLSMKAAFGKVWKLEQTGGSIIGGTFKAIKERSSNPKPPRDPRLPTPKGQTVGSFRKGLRMLPDAICERLGSKVKLSWKLSSITKSEKGGYLLTYETPEGVVSLRSRSIVMTVPSYVASNILRPLSVAAADALSSFYYPPVAAVTISYPQEAIRDERLVDGELKGFGQLHPRSQGVETLGTIYSSSLFPNRAPNGRVLLLNYIGGATNTEIVSKTESQLVEAVDRDLRKMLIKPKAQDPFVTGVRVWPQAIPQFLVGHLDTLGTAKTALSDNGHDGLFLGGNYVSGVALGRCVEGAYEIASEVTGFLSQYAYK

SEQ ID NO: 14 - protein, 553 aa, Artificial sequence
  Amino-acid sequence of PPO1 form wild-type tobacco (NtPPO1)
MTTTPIANHPNVFTHRSPPSSSSSSPSAFLTRTSFLPFSSICKRNSVNCTGWRTRCSVAKDYTVPSSAVDGGPAAELDCVIVGAGISGLCIAQVMSANYPNLMVTEARDRAGGNITTVERDGYLWEEGPNSFQPSDPMLTMAVDCGLKDDLVLGDPNAPRFVLWKGKLRPVPSKLTDLPFFDLMSIPGKLRAGFGAIGLRPSPPGHEESVEQFVRRNLGGEVFERLIEPFCSGVYAGDPSKLSMKAAFGKVWKLEETGGSIIGGTFKAIKERSSTPKAPRDPRLPKPKGQTVGSFRKGLRMLPDAISARLGSKLKLSWKLSSITKSEKGGYRLTYETPEGVVSLQSRSIVMTVPSYVASNILRPLSVAAADALSNFYYPPVGAVTISYPQEAIRDERLVDGELKGFGQLHPRTQGVETLGTIYSSSLFPNRAPKGRVLLLNYIGGAKNPEILSKTESQLVEVVDRDLRKMLIKPKAQDPLVVGVRVWPQAIPQFLVGHLDTLSTAKAAMSDNGLEGLFLGGNYVSGVALGRCVEGAYEVASEVTGFLPRYAYK

SEQ ID NO: 15 - protein, 537 aa, Artificial sequence
  Amino-acid sequence of PPO1 from wild-type Arabidopsis thaliana (AtPPO1)
MELSLLRPTTQSLLPSFSKPNLRLNVYKPLRLRCSVAGGPTVGSSKIEGGGGTTITTDCVIVGGGISGLCIAQALATKHPDAAPNLIVTEAKDRVGGNIITREENGFLWEEGPNSFQPSDPMLTMVVDSGLKDDLVLGDPTAPRFVLWNGKLRPVPSKLTDLPFFDLMSIGGKIRAGFGALGIRPSPPGREESVEEFVRRNLGDEVFERLIEPFCSGVYAGDPSKLSMKAAFGKVWKLEQNGGSIIGGTFKAIQERKNAPKAERDPRLPKPQGQTVGSFRKGLRMLPEAISARLGSKVKLSWKLSGITKLESGGYNLTYETPDGLVSVQSKSVVMTVPSHVASGLLRPLSESAANALSKLYYPPVAAVSISYPKEAIRTECLIDGELKGFGQLHPRTQGVETLGTIYSSSLFPNRAPPGRILLLNYIGGSTNTGILSKSEGELVEAVDRDLRKMLIKPNSTDPLKLGVRVWPQAIPQFLVGHFDILDTAKSSLTSSGYEGLFLGGNYVAGVALGRCVEGAYETAIEVNNFMSRYAYK

SEQ ID NO: 16 - protein, 539 aa, Artificial sequence
  Amino-acid sequence of PPO1 from wild-type upland cotton (GhPPO1)
MTALIDLSLLRSSPSVSPFSIPHHQHPPRFRKPFKLRCSLAEGPTISSSKIDGGESSIADCVIVGGGISGLCIAQALATKHRDVASNVIVTEARDRVGGNITTVERDGYLWEEGPNSFQPSDPILTMAVDSGLKDDLVLGDPNAPRFVLWEGKLRPVPSKPTDLPFFDLMSIAGKLRAGFGAIGIRPPPPGYEESVEEFVRRNLGAEVFERFIEPFCSGVYAGDPSKLSMKAAFGRVWKLEEIGGSIIGGTFKTIQERNKTPKPPRDPRLPKPKGQTVGSFRKGLTMLPEAIANSLGSNVKLSWKLSSITKLGNGGYNLTFETPEGMVSLQSRSVVMTIPSHVASNLLHPLSAAAADALSQFYYPPVASVTVSYPKEAIRKECLIDGELKGFGQLHPRSQGIETLGTIYSSSLFPNRAPSGRVLLLNYIGGATNTGILSKTEGELVEAVDRDLRKMLINPNAKDPLVLGVRVWPKAIPQFLVGHLDLLDSAKMALRDSGFHGLFLGGNYVSGVALGRCVEGAYEVAAEVKEFLSQYAYK

SEQ ID NO: 17 - protein, 538 aa, Artificial sequence
  Amino-acid sequence of PPO1 from wild-type radish (RsPPO1)
MDLSLLRPQPFLSPFSNPFPRSRPYYKPLNLHCSVSGGSVVGSSTIEGGGGGGKTVAADCVIVGGGISGLCIAQALVTKHPDAAKNVIVTEAKDRVGGNIITREEQGFLWEEGPNSFQPSDPMLTMVVDSGLKDDLVLGDPTAPRFVLWNGKLRPVPSKLTDLPFFDLMSIRGKIRAGFGAIGIRPSPPGREESVEEFVRRNLGDEVFERLIEPFCSGVYAGDPAKLSMKAAFGKVWKLEENGGSIIGGAFKAIQARNKAPKTTRDPRLPKPKGQTVGSFRKGLTMLPEAISARLGNKVKVSWKLSSITKLANGEYSLTYETPEGIVTVQSKSVVMTVPSHVASSLLRPLSDSAAEALSKLYYPPVAAVSISYPKEAIRSECLIDGELKGFGQLHPRTQKVETLGTIYSSSLFPNRAPPGRVLLLNYIGGTTNTGILSKSEGELVEAVDRDLRKMLIKPSSTDPLVLGVRVWPQAIPQFLIGHIDLVDAAKASLSSSGHEGIFLGGNYVAGVALGRCVECAYETATQVNDFMSRYTYK

SEQ ID NO: 18 - protein, 535 aa, Artificial sequence
  Amino-acid sequence of PPO1 from wild-type foxtail millet (SiPPO1)
MVAAAMATAPSAGVPPLRGTRGPARFRIRGVSVRCAAVAGGAAEAPASAGARVSADCVVVGGGISGLCTAQALATKHGVGDVLVTEARARPGGNITTVERPDEGYLWEEGPNSFQPSDPVLTMAVDSGLKDDLVFGDPNAPRFVLWEGKLRPVPSKPADLPFFDLMSIPGKLRAGFGALGIRPPPPGREESVEEFVRRNLGAEVFERLIEPFCSGVYAGDPSKLSMKAAFGKVWRLEEAGGSIIGGTIKTIQERGKNPKPPRDPRLPTPKGQTVASFRKGLAMLPNAITSSLGSKVKLSWKLTSITKSDGMGYVLVYETPEGVVSVQAKSVIMTIPSYVASDILRPLSSDAADALSRFYYPPVAAVTISYPKEAIRKECLIDGELQGFGQLHPRSQGVETLGTIYSSSLFPNRAPAGRVLLLNYIGGATNTGIVSKSASELVEAVDRDLRKMLINPSAVDPLVLGVRVWPQAIPQFLVGHLDLLEAAKSSLDRGGYDGLFLGGNYVAGVALGRCVEGAYESASQISDFLTKYAYK

SEQ ID NO: 19 - protein, 537 aa, Artificial sequence
  Amino-acid sequence of PPO1 form wild-type cabbage (BoPPO1)
MDLSLLRPQPFLSPFSNPFPRSRPYKPPNLRCSVSGGSVVGGSSTIEGGGGGKTVAADCVIVGGGISGLCIAQALVTKHPDAAKSVMVTEAKDRVGGNIITREEQGFLWEEGPNSFQPSDPMLTMVVDSGLKDDLVLGDPTAPRFVLWNGKLRPVPSKLTDLPFFDLMSIGGKIRAGFGAIGIRPSPPGREESVEEFVRRNLGDEVFERLIEPFCSGVYAGDPAKLSMKAAFGKVWKLEENGGSIIGGAFKAIQARNKAPKTTRDPRLPKPKGQTVGSFRKGLTMLPEAISARLGDKVKVSWKLSSISKLPSGGYSLTYETPEGIVTVQSKSVVMTVPSHVASSLLRPLSDSAAEALSKLYYPPVAAVSISYLKEAIRSECLIDGELKGFGQLHPRTQKVETLGTIYSSSLFPNRAPPGRVLLLNYIGGATNTGILSKSEGELVEAVDRDLRKMLIMPSSTDPLVLGVKVWPQAIPQFLIGHIDLVDAAKASLSSSGHEGLFLGGNYVAGVALGRCVEGAYETATQVNDFMSRYAYK

SEQ ID NO: 20 - protein, 536 aa, Artificial sequence
  Amino-acid sequence of PPO1 from rice mutant (OsPPO1 L423S)
MAAAAAAMATATSATAAPPLRIRDAARRTRRRGHVRCAVASGAAEAPAAPGARVSADCVVVGGGISGLCTAQALATKHGVGDVLVTEARARPGGNITTAERAGEGYLWEEGPNSFQPSDPVLTMAVDSGLKDDLVFGDPNAPRFVLWEGKLRPVPSKPGDLPFFDLMSIPGKLRAGLGALGVRAPPPGREESVEDFVRRNLGAEVFERLIEPFCSGVYAGDPSKLSMKAAFGKVWRLEDTGGSIIGGTIKTIQERGKNPKPPRDPRLPTPKGQTVASFRKGLTMLPDAITSRLGSKVKLSWKLTSITKSDNKGYALVYETPEGVVSVQAKTVVMTIPSYVASDILRPLSSDAADALSIFYYPPVAAVTVSYPKEAIRKECLIDGELQGFGQLHPRSQGVETLGTIYSSSLFPNRAPAGRVLLSNYIGGSTNTGIVSKTESELVEAVDRDLRKMLINPKAVDPLVLGVRVWPQAIPQFLIGHLDHLEAAKSALGKGGYDGLFLGGNYVAGVALGRCVEGAYESASQISDYLTKYAYK

SEQ ID NO: 21 - protein, 536 aa, Artificial sequence
  Amino-acid sequence of PPO1 from rice mutant (OsPPO1 L423I)
MAAAAAAMATATSATAAPPLRIRDAARRTRRRGHVRCAVASGAAEAPAAPGARVSADCVVVGGGISGLCTAQALATKHGVGDVLVTEARARPGGNITTAERAGEGYLWEEGPNSFQPSDPVLTMAVDSGLKDDLVFGDPNAPRFVLWEGKLRPVPSKPGDLPFFDLMSIPGKLRAGLGALGVRAPPPGREESVEDFVRRNLGAEVFERLIEPFCSGVYAGDPSKLSMKAAFGKVWRLEDTGGSIIGGTIKTIQERGKNPKPPRDPRLPTPKGQTVASFRKGLTMLPDAITSRLGSKVKLSWKLTSITKSDNKGYALVYETPEGVVSVQAKTVVMTIPSYVASDILRPLSSDAADALSIFYYPPVAAVTVSYPKEAIRKECLIDGELQGFGQLHPRSQGVETLGTIYSSSLFPNRAPAGRVLLINYIGGSTNTGIVSKTESELVEAVDRDLRKMLINPKAVDPLVLGVRVWPQAIPQFLIGHLDHLEAAKSALGKGGYDGLFLGGNYVAGVALGRCVEGAYESASQISDYLTKYAYK

SEQ ID NO: 22 - protein, 536 aa, Artificial sequence
  Amino-acid sequence of PPO1 from rice mutant (OsPPO1 L423G)
MAAAAAAMATATSATAAPPLRIRDAARRTRRRGHVRCAVASGAAEAPAAPGARVSADCVVVGGGISGLCTAQALATKHGVGDVLVTEARARPGGNITTAERAGEGYLWEEGPNSFQPSDPVLTMAVDSGLKDDLVFGDPNAPRFVLWEGKLRPVPSKPGDLPFFDLMSIPGKLRAGLGALGVRAPPPGREESVEDFVRRNLGAEVFERLIEPFCSGVYAGDPSKLSMKAAFGKVWRLEDTGGSIIGGTIKTIQERGKNPKPPRDPRLPTPKGQTVASFRKGLTMLPDAITSRLGSKVKLSWKLTSITKSDNKGYALVYETPEGVVSVQAKTVVMTIPSYVASDILRPLSSDAADALSIFYYPPVAAVTVSYPKEAIRKECLIDGELQGFGQLHPRSQGVETLGTIYSSSLFPNRAPAGRVLLGNYIGGSTNTGIVSKTESELVEAVDRDLRKMLINPKAVDPLVLGVRVWPQAIPQFLIGHLDHLEAAKSALGKGGYDGLFLGGNYVAGVALGRCVEGAYESASQISDYLTKYAYK

SEQ ID NO: 23 - protein, 536 aa, Artificial sequence
  Amino-acid sequence of PPO1 from rice mutant (OsPPO1 Y425M)
MAAAAAAMATATSATAAPPLRIRDAARRTRRRGHVRCAVASGAAEAPAAPGARVSADCVVVGGGISGLCTAQALATKHGVGDVLVTEARARPGGNITTAERAGEGYLWEEGPNSFQPSDPVLTMAVDSGLKDDLVFGDPNAPRFVLWEGKLRPVPSKPGDLPFFDLMSIPGKLRAGLGALGVRAPPPGREESVEDFVRRNLGAEVFERLIEPFCSGVYAGDPSKLSMKAAFGKVWRLEDTGGSIIGGTIKTIQERGKNPKPPRDPRLPTPKGQTVASFRKGLTMLPDAITSRLGSKVKLSWKLTSITKSDNKGYALVYETPEGVVSVQAKTVVMTIPSYVASDILRPLSSDAADALSIFYYPPVAAVTVSYPKEAIRKECLIDGELQGFGQLHPRSQGVETLGTIYSSSLFPNRAPAGRVLLLNMIGGSTNTGIVSKTESELVEAVDRDLRKMLINPKAVDPLVLGVRVWPQAIPQFLIGHLDHLEAAKSALGKGGYDGLFLGGNYVAGVALGRCVEGAYESASQISDYLTKYAYK

SEQ ID NO: 24 - protein, 536 aa, Artificial sequence
  Amino-acid sequence of PPO1 from rice mutant (OsPPO1 Y425I)
MAAAAAAMATATSATAAPPLRIRDAARRTRRRGHVRCAVASGAAEAPAAPGARVSADCVVVGGGISGLCTAQALATKHGVGDVLVTEARARPGGNITTAERAGEGYLWEEGPNSFQPSDPVLTMAVDSGLKDDLVFGDPNAPRFVLWEGKLRPVPSKPGDLPFFDLMSIPGKLRAGLGALGVRAPPPGREESVEDFVRRNLGAEVFERLIEPFCSGVYAGDPSKLSMKAAFGKVWRLEDTGGSIIGGTIKTIQERGKNPKPPRDPRLPTPKGQTVASFRKGLTMLPDAITSRLGSKVKLSWKLTSITKSDNKGYALVYETPEGVVSVQAKTVVMTIPSYVASDILRPLSSDAADALSIFYYPPVAAVTVSYPKEAIRKECLIDGELQGFGQLHPRSQGVETLGTIYSSSLFPNRAPAGRVLLLNIIGGSTNTGIVSKTESELVEAVDRDLRKMLINPKAVDPLVLGVRVWPQAIPQFLIGHLDHLEAAKSALGKGGYDGLFLGGNYVAGVALGRCVEGAYESASQISDYLTKYAYK

SEQ ID NO: 25 - protein, 536 aa, Artificial sequence
  Amino-acid sequence of PPO1 from rice mutant (OsPPO1 Y425V)
MAAAAAAMATATSATAAPPLRIRDAARRTRRRGHVRCAVASGAAEAPAAPGARVSADCVVVGGGISGLCTAQALATKHGVGDVLVTEARARPGGNITTAERAGEGYLWEEGPNSFQPSDPVLTMAVDSGLKDDLVFGDPNAPRFVLWEGKLRPVPSKPGDLPFFDLMSIPGKLRAGLGALGVRAPPPGREESVEDFVRRNLGAEVFERLIEPFCSGVYAGDPSKLSMKAAFGKVWRLEDTGGSIIGGTIKTIQERGKNPKPPRDPRLPTPKGQTVASFRKGLTMLPDAITSRLGSKVKLSWKLTSITKSDNKGYALVYETPEGVVSVQAKTVVMTIPSYVASDILRPLSSDAADALSIFYYPPVAAVTVSYPKEAIRKECLIDGELQGFGQLHPRSQGVETLGTIYSSSLFPNRAPAGRVLLLNVIGGSTNTGIVSKTESELVEAVDRDLRKMLINPKAVDPLVLGVRVWPQAIPQFLIGHLDHLEAAKSALGKGGYDGLFLGGNYVAGVALGRCVEGAYESASQISDYLTKYAYK

SEQ ID NO: 26 - protein, 536 aa, Artificial sequence
  Amino-acid sequence of PPO1 from rice mutant (OsPPO1 L423S/Y425I)
MAAAAAAMATATSATAAPPLRIRDAARRTRRRGHVRCAVASGAAEAPAAPGARVSADCVVVGGGISGLCTAQALATKHGVGDVLVTEARARPGGNITTAERAGEGYLWEEGPNSFQPSDPVLTMAVDSGLKDDLVFGDPNAPRFVLWEGKLRPVPSKPGDLPFFDLMSIPGKLRAGLGALGVRAPPPGREESVEDFVRRNLGAEVFERLIEPFCSGVYAGDPSKLSMKAAFGKVWRLEDTGGSIIGGTIKTIQERGKNPKPPRDPRLPTPKGQTVASFRKGLTMLPDAITSRLGSKVKLSWKLTSITKSDNKGYALVYETPEGVVSVQAKTVVMTIPSYVASDILRPLSSDAADALSIFYYPPVAAVTVSYPKEAIRKECLIDGELQGFGQLHPRSQGVETLGTIYSSSLFPNRAPAGRVLLSNIIGGSTNTGIVSKTESELVEAVDRDLRKMLINPKAVDPLVLGVRVWPQAIPQFLIGHLDHLEAAKSALGKGGYDGLFLGGNYVAGVALGRCVEGAYESASQISDYLTKYAYK

SEQ ID NO: 27 - protein, 537 aa, Artificial sequence
  Amino-acid sequence of PPO1 from corn mutant (ZmPPO1 L424T/Y426V)
MVAATATATAMATAASPLLNGTRIPARLRHRGLSVRCAAVAGGAAEAPASTGARLSADCVVVGGGISGLCTAQALATRHGVGDVLVTEARARPGGNITTVERPEEGYLWEEGPNSFQPSDPVLTMAVDSGLKDDLVFGDPNAPRFVLWEGKLRPVPSKPADLPFFDLMSIPGKLRAGLGALGIRPPPPGREESVEEFVRRNLGAEVFERLIEPFCSGVYAGDPSKLSMKAAFGKVWRLEETGGSIIGGTIKTIQERSKNPKPPRDARLPKPKGQTVASFRKGLAMLPNAITSSLGSKVKLLWKLTSITKSDDKGYVLEYETPEGVVSVQAKSVIMTIPSYVASNILRPLSSDAADALSRFYYPPVAAVTVSYPKEAIRKECLIDGELQGFGQLHPRSQGVETLGTIYSSSLFPNRAPDGRVLLTNVIGGATNTGIVSKTESELVEAVDRDLRKMLINSTAVDPLVLGVRVWPQAIPQFLVGHLDLLEAAKAALDRGGYDGLFLGGNYVAGVALGRCVEGAYESASQISDFLTKYAYK

SEQ ID NO: 28 - protein, 537 aa, Artificial sequence
  Amino-acid sequence of PPO1 form corn mutant (ZmPPO1 L424S/Y426V)
MVAATATATAMATAASPLLNGTRIPARLRHRGLSVRCAAVAGGAAEAPASTGARLSADCVVVGGGISGLCTAQALATRHGVGDVLVTEARARPGGNITTVERPEEGYLWEEGPNSFQPSDPVLTMAVDSGLKDDLVFGDPNAPRFVLWEGKLRPVPSKPADLPFFDLMSIPGKLRAGLGALGIRPPPPGREESVEEFVRRNLGAEVFERLIEPFCSGVYAGDPSKLSMKAAFGKVWRLEETGGSIIGGTIKTIQERSKNPKPPRDARLPKPKGQTVASFRKGLAMLPNAITSSLGSKVKLLWKLTSITKSDDKGYVLEYETPEGVVSVQAKSVIMTIPSYVASNILRPLSSDAADALSRFYYPPVAAVTVSYPKEAIRKECLIDGELQGFGQLHPRSQGVETLGTIYSSSLFPNRAPDGRVLLSNVIGGATNTGIVSKTESELVEAVDRDLRKMLINSTAVDPLVLGVRVWPQAIPQFLVGHLDLLEAAKAALDRGGYDGLFLGGNYVAGVALGRCVEGAYESASQISDFLTKYAYK

SEQ ID NO: 29 - protein, 537 aa, Artificial sequence
  Amino-acid sequence of PPO1 from corn mutant (ZmPPO1 L424V/Y426L)
MVAATATATAMATAASPLLNGTRIPARLRHRGLSVRCAAVAGGAAEAPASTGARLSADCVVVGGGISGLCTAQALATRHGVGDVLVTEARARPGGNITTVERPEEGYLWEEGPNSFQPSDPVLTMAVDSGLKDDLVFGDPNAPRFVLWEGKLRPVPSKPADLPFFDLMSIPGKLRAGLGALGIRPPPPGREESVEEFVRRNLGAEVFERLIEPFCSGVYAGDPSKLSMKAAFGKVWRLEETGGSIIGGTIKTIQERSKNPKPPRDARLPKPKGQTVASFRKGLAMLPNAITSSLGSKVKLLWKLTSITKSDDKGYVLEYETPEGVVSVQAKSVIMTIPSYVASNILRPLSSDAADALSRFYYPPVAAVTVSYPKEAIRKECLIDGELQGFGQLHPRSQGVETLGTIYSSSLFPNRAPDGRVLLVNLIGGATNTGIVSKTESELVEAVDRDLRKMLINSTAVDPLVLGVRVWPQAIPQFLVGHLDLLEAAKAALDRGGYDGLFLGGNYVAGVALGRCVEGAYESASQISDFLTKYAYK

SEQ ID NO: 30 - protein, 537 aa, Artificial sequence
  Amino-acid sequence of PPO1 from corn mutant (ZmPPO1 L424W/Y426L)
MVAATATATAMATAASPLLNGTRIPARLRHRGLSVRCAAVAGGAAEAPASTGARLSADCVVVGGGISGLCTAQALATRHGVGDVLVTEARARPGGNITTVERPEEGYLWEEGPNSFQPSDPVLTMAVDSGLKDDLVFGDPNAPRFVLWEGKLRPVPSKPADLPFFDLMSIPGKLRAGLGALGIRPPPPGREESVEEFVRRNLGAEVFERLIEPFCSGVYAGDPSKLSMKAAFGKVWRLEETGGSIIGGTIKTIQERSKNPKPPRDARLPKPKGQTVASFRKGLAMLPNAITSSLGSKVKLLWKLTSITKSDDKGYVLEYETPEGVVSVQAKSVIMTIPSYVASNILRPLSSDAADALSRFYYPPVAAVTVSYPKEAIRKECLIDGELQGFGQLHPRSQGVETLGTIYSSSLFPNRAPDGRVLLWNLIGGATNTGIVSKTESELVEAVDRDLRKMLINSTAVDPLVLGVRVWPQAIPQFLVGHLDLLEAAKAALDRGGYDGLFLGGNYVAGVALGRCVEGAYESASQISDFLTKYAYK

SEQ ID NO: 31 - protein, 537 aa, Artificial sequence
  Amino-acid sequence of PPO1 form corn mutant (ZmPPO1 L424S/Y426I)
MVAATATATAMATAASPLLNGTRIPARLRHRGLSVRCAAVAGGAAEAPASTGARLSADCVVVGGGISGLCTAQALATRHGVGDVLVTEARARPGGNITTVERPEEGYLWEEGPNSFQPSDPVLTMAVDSGLKDDLVFGDPNAPRFVLWEGKLRPVPSKPADLPFFDLMSIPGKLRAGLGALGIRPPPPGREESVEEFVRRNLGAEVFERLIEPFCSGVYAGDPSKLSMKAAFGKVWRLEETGGSIIGGTIKTIQERSKNPKPPRDARLPKPKGQTVASFRKGLAMLPNAITSSLGSKVKLLWKLTSITKSDDKGYVLEYETPEGVVSVQAKSVIMTIPSYVASNILRPLSSDAADALSRFYYPPVAAVTVSYPKEAIRKECLIDGELQGFGQLHPRSQGVETLGTIYSSSLFPNRAPDGRVLLSNIIGGATNTGIVSKTESELVEAVDRDLRKMLINSTAVDPLVLGVRVWPQAIPQFLVGHLDLLEAAKAALDRGGYDGLFLGGNYVAGVALGRCVEGAYESASQISDFLTKYAYK

SEQ ID NO: 32 - protein, 537 aa, Artificial sequence
  Amino-acid sequence of PPO1 from oilseed rape mutant (BnPPO1-C5 L424S/Y426I)
MDLSLLRPQPFLSPFSNPFPRSRPYKPPNLRCSVSGGSVVGGSSTIEGGRGGKTVAADCVIVGGGISGLCIAQALVTKHPDAAKSVMVTEAKDRVGGNIITREEQGFLWEEGPNSFQPSDPMLTMVVDSGLKDDLVLGDPTAPRFVLWNGKLRPVPSKLTDLPFFDLMSIGGKIRAGFGAIGIRPSPPGREESVEEFVRRNLGDEVFERLIEPFCSGVYAGDPAKLSMKAAFGKVWKLEENGGSIIGGAFKAIQARNKAPKTTRDPRLPKPKGQTVGSFRKGLTMLPDAISARLGDKVKVSWKLSSISKLPSGGYSLTYETPEGIVTVQSKSVVMTVPSHVASSLLRPLSDSAAEALSKLYYPPVAAVSISYPKEAIRSECLIDGELKGFGQLHPRTQKVETLGTIYSSSLFPNRAPPGRVLLSNIIGGATNTGILSKSEGELVEAVDRDLRKMLIKPSSTDPLVLGVKVWPQAIPQFLIGHIDLVDAAKASLSSSGHEGLFLGGNYVAGVALGRCVEGAYETATQVNDFMSRYAYK

SEQ ID NO: 33 - protein, 536 aa, Artificial sequence
  Amino-acid sequence of PPO1 from oilseed rape mutant (BnPPO1-A10 L423S/Y425I)
MDLSLLRPQPFLSPFSNPFPRSRPYKPLNLRCSVSGGSVVGSSTIEGGGGGKTVTADCVIVGGGISGLCIAQALVTKHPDAAKNVMVTEAKDRVGGNIITREEQGFLWEEGPNSFQPSDPMLTMVVDSGLKDDLVLGDPTAPRFVLWNGKLRPVPSKLTDLPFFDLMSIGGKIRAGFGAIGIRPSPPGREESVEEFVRRNLGDEVFERLIEPFCSGVYAGDPAKLSMKAAFGKVWKLEENGGSIIGGAFKAIQAKNKAPKTTRDPRLPKPKGQTVGSFRKGLTMLPEAISARLGDKVKVSWKLSSITKLASGEYSLTYETPEGIVTVQSKSVVMTVPSHVASSLLRPLSDSAAEALSKLYYPPVAAVSISYAKEAIRSECLIDGELKGFGQLHPRTQKVETLGTIYSSSLFPNRAPPGRVLLSNIIGGATNTGILSKSEGELVEAVDRDLRKMLIKPSSTDPLVLGVKLWPQAIPQFLIGHIDLVDAAKASLSSSGHEGLFLGGNYVAGVALGRCVEGAYETATQVNDFMSRYAYK

SEQ ID NO: 34 - protein, 558 aa, Artificial sequence
  Amino-acid sequence of PPO1 from peanut mutant (AhPPO1-A L445S/Y447I)
MPAMLTLPNDTVFLQNTMHSPTSSFSPHSPLIIPFPSPCRHPSTTKFPLIRCSLAGESSTASPAKPAALPRSAVGASVDCVVVGGGISGLCIAQALSTKHAKAAANVVVTEARDRVGGNITTIERDGYLWEEGPNSFQPSDPMLTMVVDSGLKDELVLGDPNAPRFVLWNGELRPVPGKPTDLPFFDLMSFGGKLRAGFGALGIRPPPPGHEESVEEFVRRNLGDEVFERLIEPFCSGVYAGDPSKLSMKAAFGKVWRLEQNGGSIIGGTFKAIQERKSTSKPPRDPRLPTPKGQTVGSFRKGLTMLPEAISAKLGNKVKLSWKLLGISKLDSGEYSLTYDTPEGVVSLQTKSVVMTIPSHVASTLLRSISDAAADALSKFYYPPVAAVSVSYPKEAIRSECLIDGELKGFGQLHPRTQGVETLGTIYSSSLFPNRAPDGRVLLSNIIGGATNPGILSKTDSELVEAVDRDLRKMLINPNAGDPFALGVRVWPQAIPQFLVGHLDLLDIAKSSLKNTGFEGLFLGGNYVSGVALGRCVEGAYEIAAEVDDFLAQKVYK

SEQ ID NO: 35 - protein, 552 aa, Artificial sequence
  Amino-acid sequence of PPO1 from peanut mutant (AhPPO1-B L439S/Y441I)
MSAMLTLPNDTVFLQNTMHSPTSSFSPHSPLIIPFPSPCRHPSTTKFPLIRCSLAGESSTASLPRSAVGASVDCVVVGGGISGLCIAQALSTKHAKAAANVVVTEARDRVGGNITTVERDGYLWEEGPNSFQPSDPMLTMVVDSGLKDELVLGDPNAPRFVLWNGRLRPVPGKPTDLPFFDLMSFGGKLRAGFGALGIRPPPPGHEESVEEFVRRNLGDEVFERLIEPFCSGVYAGDPSKLSMKAAFGKVWRLEQNGGSIIGGTFKAIQERKSTSKPPRDPRLPTPKGQTVGSFRKGLIMLPEAISAKLGNKVKLSWKLLGISKLDSGEYSLTYDTPEGVVSLQTKSVVMTIPSHVASTLLRSISETAADALSKFYYPPVAAVSVSYPKEAIRSECLIDGELKGFGQLHPRTQGVETLGTIYSSSLFPNRAPDGRVLLSNIIGGATNPGILSKTDSELVEAVDRDLRKMLINPNAGDPFALGVRVWPQAIPQFLVGHLDLLDIAKSSLKNTGFEGLFLGGNYVSGVALGRCVEGAYEIAAEVDDFLAQKVYK

SEQ ID NO: 36 - protein, 543 aa, Artificial sequence
  Amino-acid sequence of PPO1 from soybean mutant (GmPPO1 L430S/Y432I)
MVSVFNEILFPPNQTLLRPSLHSPTSFFTSPTRKFPRSRPNPILRCSIAEESTASPPKTRDSAPVDCVVVGGGVSGLCIAQALATKHANANVVVTEARDRVGGNITTMERDGYLWEEGPNSFQPSDPMLTMVVDSGLKDELVLGDPDAPRFVLWNRKLRPVPGKLTDLPFFDLMSIGGKIRAGFGALGIRPPPPGHEESVEEFVRRNLGDEVFERLIEPFCSGVYAGDPSKLSMKAAFGKVWKLEKNGGSIIGGTFKAIQERNGASKPPRDPRLPKPKGQTVGSFRKGLTMLPDAISARLGNKVKLSWKLSSISKLDSGEYSLTYETPEGVVSLQCKTVVLTIPSYVASTLLRPLSAAAADALSKFYYPPVAAVSISYPKEAIRSECLIDGELKGFGQLHPRSQGVETLGTIYSSSLFPNRAPPGRVLLSNIIGGATNTGILSKTDSELVETVDRDLRKILINPNAQDPFVVGVRLWPQAIPQFLVGHLDLLDVAKASIRNTGFEGLFLGGNYVSGVALGRCVEGAYEVAAEVNDFLTNRVYK

SEQ ID NO: 37 - protein, 536 aa, Artificial sequence
  Amino-acid sequence of PPO1 from sorghum mutant (SbPPO1 L423S/Y425I)
MVAAAAMATAASAAAPLLNGTRRPARLRRRGLRVRCAAVAGGAAEAPASTGARLSADCVVVGGGISGLCTAQALATRHGVGEVLVTEARARPGGNITTVERPEEGYLWEEGPNSFQPSDPVLSMAVDSGLKDDLVFGDPNAPRFVLWEGKLRPVPSKPADLPFFDLMSIPGKLRAGLGALGIRPPPPGREESVEEFVRRNLGAEVFERLIEPFCSGVYAGDPSKLSMKAAFGKVWRLEEAGGSIIGGTIKTIQERGKNPKPPRDPRLPKPKGQTVASFRKGLAMLPNAITSSLGSKVKLSWKLTSITKSDGKGYVLEYETPEGVVLVQAKSVIMTIPSYVASDILRPLSGDAADALSRFYYPPVAAVTVSYPKEAIRKECLIDGELQGFGQLHPRSQGVETLGTIYSSSLFPNRAPAGRVLLSNIIGGATNTGIVSKTESELVEAVDRDLRKMLINSTAVDPLVLGVRVWPQAIPQFLVGHLDLLEVAKSALDQGGYDGLFLGGNYVAGVALGRCIEGAYESAAQIYDFLTKYAYK

SEQ ID NO: 38 - protein, 531 aa, Artificial sequence
  Amino-acid sequence of PPO1 form wheat mutant (TaPPO1-A L418S/Y420I)
MAGATMATATVTAASPLRGRVTGRPRRVRTRCAAASGATETPAAPGVRLSAECVIVGAGISGLCTAQALATRYGVSDLLVTEARDRPGGNITTVERPDEGYLWEEGPNSFQPSDPVLTMAVDSGLKDDLVFGDPNAPRFVLWEGKLRPVPSKPGDLPFFSLMSIPGKLRAGLGALGIRPPPPGREESVEEFVRRNLGAEVFERLIEPFCSGVYAGDPSKLSMKAAFGKVWRLEEIGGSIIGGTIKAIQDKGKNPKPPRDPRLPAPKGQTVASFRKGLAMLPNAIASRLGSKVKLSWKLTSITKADNQGYVLGYETPEGLVSVQAKSVIMTIPSYVASDILRPLSIDAADALSKFYYPPVAAVTVSYPKEAIRKECLIDGELQGFGQLHPRSQGVETLGTIYSSSLFPNRAPAGRVLLSNIIGGSTNTGIVSKTESDLVEAVDRDLRKMLINPRAADPLALGVRVWPQAIPQFLIGHLDRLAAAKSALGRGGYDGLFLGGNYVAGVALGRCIEGAYESASQVSDFLTKYAYK

SEQ ID NO: 39 - protein, 531 aa, Artificial sequence
  Amino-acid sequence of PPO1 from wheat mutant (TaPPO1-B L418S/Y420I)
MAGATMATATVAAASPLRGRVTGRPHRVRPRCATASSATETPAAPGVRLSAECVIVGAGISGLCTAQALATRYGVSDLLVTEARDRPGGNITTVERPDEGYLWEEGPNSFQPSDPVLTMAVDSGLKDDLVFGDPNAPRFVLWEGKLRPVPSKPGDLPFFSLMSIPGKLRAGLGALGIRPPPPGREESVEEFVRRNLGAEVFERLIEPFCSGVYAGDPSKLSMKAAFGKVWRLEEIGGSIIGGTIKAIQDKGKNPKPPRDPRLPAPKGQTVASFRKGLAMLPNAIASRLGSKVKLSWKLTSITKADNQGYVLGYETPEGLVSVQAKSVIMTIPSYVASDILRPLSIDAADALSKFYYPPVAAVTVSYPKEAIRKECLIDGELQGFGQLHPRSQGVETLGTIYSSSLFPNRAPAGRVLLSNIIGGSTNTGIVSKTESDLVGAVDRDLRKMLINPRAADPLALGVRVWPQAIPQFLIGHLDRLAAAKSALGQGGYDGLFLGGNYVAGVALGRCIEGAYESASQVSDFLTKYAYK

SEQ ID NO: 40 - protein, 531 aa, Artificial sequence
  Amino-acid sequence of PPO1 form wheat mutant (TaPPO1-D L418S/Y420I)
MAGATMATATVTAASPLRGRVTGRPRRVRPRCAAASGATETPAAPGVRLSADCVIVGAGISGLCTAQALATRYGVGDLLITEARDRPGGNITTVERPDEGYLWEEGPNSFQPSDPVLTMAVDSGLKDDLVFGDPNAPRFVLWEGKLRPVPSKPGDLPFFSLMSIPGKLRAGLGALGIRPPPPGREESVEEFVRRNLGAEVFERLIEPFCSGVYAGDPSKLSMKAAFGKVWRLEEIGGSIIGGTIKAIQDKGKNPKPPRDPRLPAPKGQTVASFRKGLAMLPNAIASRLGSKVKLSWKLTSITKADNQGYVLGYETPEGLVSVQAKSVIMTIPSYVASDILRPLSIDAADALSKFYYPPVAAVTVSYPKEAIRKECLIDGELQGFGQLHPRSQGVETLGTIYSSSLFPNRAPAGRVLLSNIIGGSTNTGIVSKTESDLVEAVDSDLRKMLINPRAADPLALGVRVWPQAIPQFLIGHLDRLAAAKSALGRGGYDGLFLGGNYVAGVALGRCIEGAYESASQVSDFLTKYAYK

SEQ ID NO: 41 - protein, 558 aa, Artificial sequence
  Amino-acid sequence of PPO1 form tomato mutant (SlPPO1 L445S/Y447I)
MTTTAVVNHPSIFTHRSPLPSPSSSSSSSPSFLFLNRTNFIPYFSTSKRSSVNCNGWRTRCSVAKNYTVPPSEVDGNQLPELDCVVVGAGISGLCIAKVISANYPNLMVTEARDRAGGNITTVERDGYLWEEGPNSFQPSDPMLTMAVDCGLKDDLVLGDPDAPRFVLWKDKLRPVPGKLTDLPFFDLMSIPGKLRAGFGAIGLRPSPPGYEESVEQFVRRNLGAEVFERLIESFCSGVYAGDPSKLSMKAAFGKVWKLEQTGGSIIGGTFKAIKERSSNPKPPRDPRLPTPKGQTVGSFRKGLRMLPDAICERLGSKVKLSWKLSSITKSDKGGYLLTYETPEGVVSLRSRSIVMTVPSYVASNILRPLSVAAADALSSFYYPPVAAVTISYPQEAIRDERLVDGELKGFGQLHPRSQGVETLGTIYSSSLFPNRAPNGRVLLSNIIGGATNTEIVSKTESQLVEAVDRDLRKMLIKPKAQDPFVTGVRVWPQAIPQFLVGHLDTLGTAKAALSDNGLDGLFLGGNYVSGVALGRCVEGAYEIASEVTGFLSQYAYK

SEQ ID NO: 42 - protein, 557 aa, Artificial sequence
  Amino-acid sequence of PPO1 form potato mutant (StPPO1 L444S/Y446I)
MTTTAVANHPSIFTHRSPLLSPSSSSSSPSFLFLNRTNFIPYFSTSKRNSVNCNGWRTRCSVAKDYTVPPSEVDGNQFPELDCVVVGAGISGLCITKVISDNYPNLMVTEARDRAGGNITTVERDGYLWEEGPNSFQPSDPMLTMAVDCGLKDDLVLGDPDAPRFVLWKDKLRPVPGKLTDLPFFDLMSIPGKLRAGFGAIGLRPSPPGYEESVEQFVRRNLGAEVFERLIEPFCSGVYAGDPSKLSMKAAFGKVWKLEQTGGSIIGGTFKAIKERSSNPKPPRDPRLPTPKGQTVGSFRKGLRMLPDAICERLGSKVKLSWKLSSITKSEKGGYLLTYETPEGVVSLRSRSIVMTVPSYVASNILRPLSVAAADALSSFYYPPVAAVTISYPQEAIRDERLVDGELKGFGQLHPRSQGVETLGTIYSSSLFPNRAPNGRVLLSNIIGGATNTEIVSKTESQLVEAVDRDLRKMLIKPKAQDPFVTGVRVWPQAIPQFLVGHLDTLGTAKTALSDNGHDGLFLGGNYVSGVALGRCVEGAYEIASEVTGFLSQYAYK

SEQ ID NO: 43 - protein, 553 aa, Artificial sequence
  Amino-acid sequence of PPO1 from tobacco mutant (NtPPO1 L440S/Y442I)
MTTTPIANHPNVFTHRSPPSSSSSSPSAFLTRTSFLPFSSICKRNSVNCTGWRTRCSVAKDYTVPSSAVDGGPAAELDCVIVGAGISGLCIAQVMSANYPNLMVTEARDRAGGNITTVERDGYLWEEGPNSFQPSDPMLTMAVDCGLKDDLVLGDPNAPRFVLWKGKLRPVPSKLTDLPFFDLMSIPGKLRAGFGAIGLRPSPPGHEESVEQFVRRNLGGEVFERLIEPFCSGVYAGDPSKLSMKAAFGKVWKLEETGGSIIGGTFKAIKERSSTPKAPRDPRLPKPKGQTVGSFRKGLRMLPDAISARLGSKLKLSWKLSSITKSEKGGYRLTYETPEGVVSLQSRSIVMTVPSYVASNILRPLSVAAADALSNFYYPPVGAVTISYPQEAIRDERLVDGELKGFGQLHPRTQGVETLGTIYSSSLFPNRAPKGRVLLSNIIGGAKNPEILSKTESQLVEVVDRDLRKMLIKPKAQDPLVVGVRVWPQAIPQFLVGHLDTLSTAKAAMSDNGLEGLFLGGNYVSGVALGRCVEGAYEVASEVTGFLPRYAYK

SEQ ID NO: 44 - protein, 536 aa, Artificial sequence
  Amino-acid sequence of PPO1 form Arabidopsis thaliana mutant (AtPPO1 L423S/Y425I)
MELSLLRPTTQSLLPSFSKPNLRLNVYKPLRLRCSVAGGPTVGSSKIEGGGGTTITTDCVIVGGGISGLCIAQALATKHPDAAPNLIVTEAKDRVGGNIITREENGFLWEEGPNSFQPSDPMLTMVVDSGLKDDLVLGDPTAPRFVLWNGKLRPVPSKLTDLPFFDLMSIGGKIRAGFGALGIRPSPPGREESVEEFVRRNLGDEVFERLIEPFCSGVYAGDPSKLSMKAAFGKVWKLEQNGGSIIGGTFKAIQERKNAPKAERDPRLPKPQGQTVGSFRKGLRMLPEAISARLGSKVKLSWKLSGITLESGGYNLTYETPDGLVSVQSKSVVMTVPSHVASGLLRPLSESAANALSKLYYPPVAAVSISYPKEAIRTECLIDGELKGFGQLHPRTQGVETLGTIYSSSLFPNRAPPGRILLSNIIGGSTNTGILSKSEGELVEAVDRDLRKMLIKPNSTDPLKLGVRVWPQAIPQFLVGHFDILDTAKSSLTSSGYEGLFLGGNYVAGVALGRCVEGAYETAIEVNNFMSRYAYK

SEQ ID NO: 45 - protein, 539 aa, Artificial sequence
  Amino-acid sequence of PPO1 from upland cotton mutant (GhPPO1 L426S/Y428I)
MTALIDLSLLRSSPSVSPFSIPHHQHPPRFRKPFKLRCSLAEGPTISSSKIDGGESSIADCVIVGGGISGLCIAQALATKHRDVASNVIVTEARDRVGGNITTVERDGYLWEEGPNSFQPSDPILTMAVDSGLKDDLVLGDPNAPRFVLWEGKLRPVPSKPTDLPFFDLMSIAGKLRAGFGAIGIRPPPPGYEESVEEFVRRNLGAEVFERFIEPFCSGVYAGDPSKLSMKAAFGRVWKLEEIGGSIIGGTFKTIQERNKTPKPPRDPRLPKPKGQTVGSFRKGLTMLPEAIANSLGSNVKLSWKLSSITKLGNGGYNLTFETPEGMVSLQSRSVVMTIPSHVASNLLHPLSAAAADALSQFYYPPVASVTVSYPKEAIRKECLIDGELKGFGQLHPRSQGIETLGTIYSSSLFPNRAPSGRVLLSNIIGGATNTGILSKTEGELVEAVDRDLRKMLINPNAKDPLVLGVRVWPKAIPQFLVGHLDLLDSAKMALRDSGFHGLFLGGNYVSGVALGRCVEGAYEVAAEVKEFLSQYAYK

SEQ ID NO: 46 - protein, 538 aa, Artificial sequence
  Amino-acid sequence of PPO1 from radish mutant (RsPPO1 L425S/Y427I)
MDLSLLRPQPFLSPFSNPFPRSRPYYKPLNLHCSVSGGSVVGSSTIEGGGGGGKTVAADCVIVGGGISGLCIAQALVTKHPDAAKNVIVTEAKDRVGGNIITREEQGFLWEEGPNSFQPSDPMLTMVVDSGLKDDLVLGDPTAPRFVLWNGKLRPVPSKLTDLPFFDLMSIRGKIRAGFGAIGIRPSPPGREESVEEFVRRNLGDEVFERLIEPFCSGVYAGDPAKLSMKAAFGKVWKLEENGGSIIGGAFKAIQARNKAPKTTRDPRLPKPKGQTVGSFRKGLTMLPEAISARLGNKVKVSWKLSSITKLANGEYSLTYETPEGIVTVQSKSVVMTVPSHVASSLLRPLSDSAAEALSKLYYPPVAAVSISYPKEAIRSECLIDGELKGFGQLHPRTQKVETLGTIYSSSLFPNRAPPGRVLLSNIIGGTTNTGILSKSEGELVEAVDRDLRKMLIKPSSTDPLVLGVRVWPQAIPQFLIGHIDLVDAAKASLSSSGHEGIFLGGNYVAGVALGRCVECAYETATQVNDFMSRYTYK

SEQ ID NO: 47 - protein, 535 aa, Artificial sequence
  Amino-acid sequence of PPO1 from foxtail millet mutant (SiPPO1 L422S/Y424I)
MVAAAMATAPSAGVPPLRGTRGPARFRIRGVSVRCAAVAGGAAEAPASAGARVSADCVVVGGGISGLCTAQALATKHGVGDVLVTEARARPGGNITTVERPDEGYLWEEGPNSFQPSDPVLTMAVDSGLKDDLVFGDPNAPRFVLWEGKLRPVPSKPADLPFFDLMSIPGKLRAGFGALGIRPPPPGREESVEEFVRRNLGAEVFERLIEPFCSGVYAGDPSKLSMKAAFGKVWRLEEAGGSIIGGTIKTIQERGKNPKPPRDPRLPTPKGQTVASFRKGLAMLPNAITSSLGSKVKLSWKLTSITKSDGMGYVLVYETPEGVVSVQAKSVIMTIPSYVASDILRPLSSDAADALSRFYYPPVAAVTISYPKEAIRKECLIDGELQGFGQLHPRSQGVETLGTIYSSSLFPNRAPAGRVLLSNIIGGATNTGIVSKSASELVEAVDRDLRKMLINPSAVDPLVLGVRVWPQAIPQFLVGHLDLLEAAKSSLDRGGYDGLFLGGNYVAGVALGRCVEGAYESASQISDFLTKYAYK

SEQ ID NO: 48 - protein, 537 aa, Artificial sequence
  Amino-acid sequence of PPO1 from cabbage mutant (BoPPO1 L424S/Y426I)
MDLSLLRPQPFLSPFSNPFPRSRPYKPPNLRCSVSGGSVVGGSSTIEGGGGGKTVAADCVIVGGGISGLCIAQALVTKHPDAAKSVMVTEAKDRVGGNIITREEQGFLWEEGPNSFQPSDPMLTMVVDSGLKDDLVLGDPTAPRFVLWNGKLRPVPSKLTDLPFFDLMSIGGKIRAGFGAIGIRPSPPGREESVEEFVRRNLGDEVFERLIEPFCSGVYAGDPAKLSMKAAFGKVWKLEENGGSIIGGAFKAIQARNKAPKTTRDPRLPKPKGQTVGSFRKGLTMLPEAISARLGDKVKVSWKLSSISKLPSGGYSLTYETPEGIVTVQSKSVVMTVPSHVASSLLRPLSDSAAEALSKLYYPPVAAVSISYLKEAIRSECLIDGELKGFGQLHPRTQKVETLGTIYSSSLFPNRAPPGRVLLSNIIGGATNTGILSKSEGELVEAVDRDLRKMLIMPSSTDPLVLGVKVWPQAIPQFLIGHIDLVDAAKASLSSSGHEGLFLGGNYVAGVALGRCVEGAYETATQVNDFMSRYAYK

SEQ ID NO: 49 - DNA, 1258 bp, Artificial sequence
  Amino-acid sequence of PPO1 from homologous replacement repair template of rice mutant (OsPPO1 L423S/Y425I)
acatgaactagtaatgattggggtgcttaaccatttgttctgcatttcctccattttcaggttgggtagcaaagtcaaactttcatggaagttgacaagcattacaaagtcagacaacaaaggatatgcattagtgtatgaaacaccagaaggggtggtctcggtgcaagctaaaactgttgtcatgaccatcccatcatatgttgctagtgatatcttgcggccactttcagtaagttatatatatttaattaactttctgttcccaaaatacactgcagcacttcattgcttcctgaggtcctcgattcatttttcggtagacaggaagtagtattcatttgcactttttaagggattaattcaacatatccactggaaatatacatatcctacacatcctgtcaacatacttgctaaacagcattttgtttgagttgactggcatctcagcagccaattactatctttaggggacaagccacattcttaataaatcctgtcggaaatcactttttgatttttatagattagtgttgtcatagaatttggcttggtgatctacttggtaaggttaactgattcacaagtcggacaatttcttcaccaatctagcagtatgtttaagtgtgttggtacttaattctaaatgtcctgcgcatggtaacatatcatatgcaaaaattcctcagtaaccgaaatttatactgtaagttttaactgtctttacactgttaattttagacatacttcttccttgcttgttcattgaacttgtttcccccttccacagagtgatgcagcagatgctctgtcaatattctattatccaccagttgctgctgtaactgtttcatatccaaaagaagcaattagaaaagaatgcttaattgacggagagctccagggtttcggccagctgcatccgcgtagtcagggagttgagactttaggtacttataggaattcaaccttattattcttctaacatataaatgaactaatctttcttgtctagtttgcatttattgtggattaagtttggttatattgttcttacaagtttgtggtattattttgtataggaacaatatatagctcatcactctttccaaatcgtgctccagctggaagggtgttactttccaacatcataggaggttctacaaatacagggattgtttccaaggtatcgctgtcaagttgtttattttgcgactatatgattacagtatcctgtttttcaactccagctgct